European Patent Application EP 4 649 948 A1, published November 19, 2025. Title: 心臓拡張機能改善剤および心臓拡張機能改善剤のスクリーニング方法. Applicant: 慶應義塾. The sequence listing filed with the application follows.

SEQUENCE LISTING (20 sequences)

SEQ ID NO: 1 - protein, 442 aa, Homo sapiens
MYQSLAMAANHGPPPGAYEAGGPGAFMHGAGAASSPVYVPTPRVPSSVLGLSYLQGGGAGSASGGASGGSSGGAASGAGPGTQQGSPGWSQAGADGAAYTPPPVSPRFSFPGTTGSLAAAAAAAAAREAAAYSSGGGAAGAGLAGREQYGRAGFAGSYSSPYPAYMADVGASWAAAAAASAGPFDSPVLHSLPGRANPAARHPNLDMFDDFSEGRECVNCGAMSTPLWRRDGTGHYLCNACGLYHKMNGINRPLIKPQRRLSASRRVGLSCANCQTTTTTLWRRNAEGEPVCNACGLYMKLHGVPRPLAMRKEGIQTRKRKPKNLNKSKTPAAPSGSESLPPASGASSNSSNATTSSSEEMRPIKTEPGLSSHYGHSSSVSQTFSVSAMSGHGPSIHPVLSALKLSPQGYASPVSQSPQTSSKQDSWNSLVLADSHGDIITA

SEQ ID NO: 2 - DNA, 1329 bp, Homo sapiens
  source 1..1329: mol_type = genomic DNA
atgtatcagagcttggccatggccgccaaccacgggccgccccccggtgcctacgaggcgggcggccccggcgccttcatgcacggcgcgggcgccgcgtcctcgccagtctacgtgcccacaccgcgggtgccctcctccgtgctgggcctgtcctacctccagggcggaggcgcgggctctgcgtccggaggcgcctcgggcggcagctccggtggggccgcgtctggtgcggggcccgggacccagcagggcagcccgggatggagccaggcgggagccgacggagccgcttacaccccgccgccggtgtcgccgcgcttctccttcccggggaccaccgggtccctggcggccgccgccgccgctgccgcggcccgggaagctgcggcctacagcagtggcggcggagcggcgggtgcgggcctggcgggccgcgagcagtacgggcgcgccggcttcgcgggctcctactccagcccctacccggcttacatggccgacgtgggcgcgtcctgggccgcagccgccgccgcctccgccggccccttcgacagcccggtcctgcacagcctgcccggccgggccaacccggccgcccgacaccccaatctcgatatgtttgacgacttctcagaaggcagagagtgtgtcaactgtggggctatgtccaccccgctctggaggcgagatgggacgggtcactatctgtgcaacgcctgcggcctctaccacaagatgaacggcatcaaccggccgctcatcaagcctcagcgccggctgtccgcctcccgccgagtgggcctctcctgtgccaactgccagaccaccaccaccacgctgtggcgccgcaatgcggagggcgagcctgtgtgcaatgcctgcggcctctacatgaagctccacggggtccccaggcctcttgcaatgcggaaagaggggatccaaaccagaaaacggaagcccaagaacctgaataaatctaagacaccagcagctccttcaggcagtgagagccttcctcccgccagcggtgcttccagcaactccagcaacgccaccaccagcagcagcgaggagatgcgtcccatcaagacggagcctggcctgtcatctcactacgggcacagcagctccgtgtcccagacgttctcagtcagtgcgatgtctggccatgggccctccatccaccctgtcctctcggccctgaagctctccccacaaggctatgcgtctcccgtcagccagtctccacagaccagctccaagcaggactcttggaacagcctggtcttggccgacagtcacggggacataatcactgcgtaa

SEQ ID NO: 3 - protein, 441 aa, Mus musculus
MYQSLAMAANHGPPPGAYEAGGPGAFMHSAGAASSPVYVPTPRVPSSVLGLSYLQGGGSAAAAGTTSGGSSGAGPSGAGPGTQQGSPGWSQAGAEGAAYTPPPVSPRFSFPGTTGSLAAAAAAAAAREAAAYGSGGGAAGAGLAGREQYGRPGFAGSYSSPYPAYMADVGASWAAAAAASAGPFDSPVLHSLPGRANPGRHPNLDMFDDFSEGRECVNCGAMSTPLWRRDGTGHYLCNACGLYHKMNGINRPLIKPQRRLSASRRVGLSCANCQTTTTTLWRRNAEGEPVCNACGLYMKLHGVPRPLAMRKEGIQTRKRKPKNLNKSKTPAGPAGETLPPSSGASSGNSSNATSSSSSSEEMRPIKTEPGLSSHYGHSSSMSQTFSTVSGHGPSIHPVLSALKLSPQGYASPVTQTSQASSKQDSWNSLVLADSHGDIITA

SEQ ID NO: 4 - DNA, 1326 bp, Mus musculus
  source 1..1326: mol_type = genomic DNA
atgtaccaaagcctggccatggccgccaaccacggccccccgcccggcgcctacgaagcaggtggccctggcgccttcatgcacagcgcgggcgccgcgtcctcgcccgtctacgtgcccactccgcgggtgccgtcctctgtgctgggcctgtcctacctgcagggcggtggcagtgccgctgcagctggaaccacctcgggtggcagctccggggccggcccgtcgggtgcagggcctgggacccagcagggtagccctggctggagccaagctggagccgagggagccgcctacaccccgccgcccgtgtccccgcgcttctctttcccggggactactgggtccctggcggccgctgccgccgctgccgcagcccgggaagctgcagcctacggcagtggcggcggggcggcgggcgctggtctggctggccgagagcagtacgggcgtccgggcttcgccggctcctactccagcccctacccagcctacatggccgacgtgggagcatcctgggccgcagccgctgccgcctctgccggccccttcgacagcccagtcctgcacagcctgcctggacgggccaaccctggaagacaccccaatctcgatatgtttgatgacttctcagaaggcagagagtgtgtcaattgtggggccatgtccaccccactctggaggcgagatgggacgggacactacctgtgcaatgcctgtggcctctatcacaagatgaacggcatcaaccggcccctcattaagcctcagcgccgcctgtccgcttcccgccgggtaggcctctcctgtgccaactgccagactaccaccaccacgctgtggcgtcgtaatgccgagggtgagcctgtatgtaatgcctgcggcctctacatgaagctccatggggttcccaggcctcttgcaatgcggaaggaggggattcaaaccagaaaacggaagcccaagaacctgaataaatctaagacgccagcaggtcctgctggtgagaccctccctccctccagtggtgcctccagcggtaactccagcaatgccactagcagcagcagcagcagtgaagagatgcgccccatcaagacagagcccgggctgtcatctcactatgggcacagcagctccatgtcccagacattcagtactgtgtccggccacgggccctccatccatccagtgctgtctgctctgaagctgtccccacaaggctatgcatctcctgtcactcagacatcgcaggccagctccaagcaggactcttggaacagcctggtcctggctgacagtcatggggacataatcaccgcgtaa

SEQ ID NO: 5 - DNA, 21 bp, synthetic construct
  source 1..21: mol_type = other DNA
cagtcagttgctcaatgtacc

SEQ ID NO: 6 - DNA, 18 bp, synthetic construct
  source 1..18: mol_type = other DNA
actggtgaaactcaccca

SEQ ID NO: 7 - DNA, 22 bp, synthetic construct
  source 1..22: mol_type = other DNA
gttcgcaagaacctgatggaca

SEQ ID NO: 8 - DNA, 22 bp, synthetic construct
  source 1..22: mol_type = other DNA
ctagagcctgttttgcacgttc

SEQ ID NO: 9 - DNA, 19 bp, synthetic construct
  source 1..19: mol_type = other DNA
ctgttcctgtacggcatgg

SEQ ID NO: 10 - DNA, 20 bp, synthetic construct
  source 1..20: mol_type = other DNA
ggcattaaagcagcgtatcc

SEQ ID NO: 11 - DNA, 20 bp, synthetic construct
  source 1..20: mol_type = other DNA
atgccctggctcacaaatac

SEQ ID NO: 12 - DNA, 20 bp, synthetic construct
  source 1..20: mol_type = other DNA
gccaacctttgttcatggca

SEQ ID NO: 13 - DNA, 20 bp, synthetic construct
  source 1..20: mol_type = other DNA
ttgccgggaagctagagtaa

SEQ ID NO: 14 - DNA, 20 bp, synthetic construct
  source 1..20: mol_type = other DNA
tttgccttcctgtttttgct

SEQ ID NO: 15 - DNA, 28 bp, synthetic construct
  source 1..28: mol_type = other DNA
tcttttctgttggacccttaccttgacc

SEQ ID NO: 16 - DNA, 30 bp, synthetic construct
  source 1..30: mol_type = other DNA
acgtcaatggaaagtccctattggcgttac

SEQ ID NO: 17 - DNA, 28 bp, synthetic construct
  source 1..28: mol_type = other DNA
tgccatgaacaaaggttggctataaaga

SEQ ID NO: 18 - DNA, 28 bp, synthetic construct
  source 1..28: mol_type = other DNA
aggatagtgcagggaaacccaaagaagt

SEQ ID NO: 19 - DNA, 20 bp, synthetic construct
  source 1..20: mol_type = other DNA
agcttgtcatcaacgggaag

SEQ ID NO: 20 - DNA, 21 bp, synthetic construct
  source 1..21: mol_type = other DNA
tttgatgttagtggggtctcg